European Patent Application EP 4 238 575 A1, published September 6, 2023. Title: METHODS OF TREATING A TRAUMATIC BRAIN INJURY. Applicant: Suzhou Yabao Pharmaceutical R&D Co Ltd. The sequence listing filed with the application follows.

SEQUENCE LISTING (1 sequence)

SEQ ID NO: 1 - protein, 317 aa, Homo sapiens
AQVLRGTVTDFPGFDERADAETLRKAMKGLGTDEESILTLLTSRSNAQRQEISAAFKTLFGRDLLDDLKSELTGKFEKLIVALMKPSRLYDAYELKHALKGAGTNEKVLTEIIASRTPEELRAIKQVYEEEYGSSLEDDWGDTSGYYQRMLWLLQANRDPDAGIDEAQVEQDAQALFQAGELKWGTDEEKFITIFGTRSVSHLRKVFDKYMTISGFQIEETIDRETSGNLEQLLLAVVKSIRSIPAYLAETLYYAMKGAGTDDHTLIRVMVSRSEIDLFNIRKEFRKNFATSLYSMIKGDTSGDYKKALLLLCGEDD